European Patent Specification EP 3 966 574 B1, published August 28, 2024. Title: Novel Ligand Assays. Applicant: Otago Innovation Limited. The sequence listing filed with the application follows.

SEQUENCE LISTING (174 sequences)

SEQ ID NO: 1 - DNA, 15 bp, Artificial
  Androgen Response Element 1 - Sense Strand
  misc_feature (7)..(9): n is a, c, g, or t
agaacannntgttct

SEQ ID NO: 2 - DNA, 15 bp, Artificial
  Androgen Response Element 1 - Antisense Strand
  misc_feature (7)..(9): n is a, c, g, or t
agaacannntgttct

SEQ ID NO: 3 - DNA, 15 bp, Artificial
  Androgen Response Element 2 - Sense Strand
  misc_feature (7)..(9): n is a, c, g, or t
ggtacannntgttct

SEQ ID NO: 4 - DNA, 15 bp, Artificial
  Androgen Response Element 2 - Antisense Strand
  misc_feature (7)..(9): n is a, c, g, or t
agaacannntgtacc

SEQ ID NO: 5 - DNA, 15 bp, Artificial
  Estrogen Response Element - Sense Strand
  misc_feature (7)..(9): n is a, c, g, or t
aggtcannntgacct

SEQ ID NO: 6 - DNA, 15 bp, Artificial
  Estrogen Response Element - Sense Strand
  misc_feature (7)..(9): n is a, c, g, or t
aggtcannntgacct

SEQ ID NO: 7 - DNA, 15 bp, Artificial
  Progesterone Response Element - Sense Strand
ggtacaaactgttct

SEQ ID NO: 8 - DNA, 15 bp, Artificial
  Progesterone Response Element - Antisense Strand
agaacagtttgtacc

SEQ ID NO: 9 - DNA, 15 bp, Artificial
  Glucocorticoid/Mineralocorticoid Response Element - Sense Strand
  misc_feature (7)..(7): n is a, c, g, or t
agaacanaatgttct

SEQ ID NO: 10 - DNA, 15 bp, Artificial
  Glucocorticoid/Mineralocorticoid Response Element - Antisense Strand
  misc_feature (9)..(9): n is a, c, g, or t
agaacattntgttct

SEQ ID NO: 11 - DNA, 15 bp, Artificial
  ARE Constructs 1 & 3 - Sense Strand
  misc_feature (1)..(1): n = g + Fluorophore
  misc_feature (7)..(9): n is a, c, g, or t
ngtacannntgttct

SEQ ID NO: 12 - DNA, 15 bp, Artificial
  ARE Construct 1 - Antisense Strand
  misc_feature (1)..(1): n = a + Fluorophore
  misc_feature (7)..(9): n is a, c, g, or t
ngaacannntgtacc

SEQ ID NO: 13 - DNA, 15 bp, Artificial
  ARE Construct 2 - Sense Strand
  misc_feature (1)..(1): n = g + Fluorophore
ngtacagcatgttct

SEQ ID NO: 14 - DNA, 15 bp, Artificial
  ARE Construct 2 - Antisense Strand
  misc_feature (1)..(1): n = a + Fluorophore
ngaacatgctgtacc

SEQ ID NO: 15 - DNA, 15 bp, Artificial
  ARE Construct 3 - Sense Strand
  misc_feature (1)..(1): n = g + Fluorophore
  misc_feature (7)..(9): n is a, c, g, or t
ngtacannntgttct

SEQ ID NO: 16 - DNA, 15 bp, Artificial
  ARE Construct 3 - Antisense Strand
  misc_feature (1)..(1): n = a + Quencher
  misc_feature (7)..(9): n is a, c, g, or t
ngaacannntgtacc

SEQ ID NO: 17 - DNA, 15 bp, Artificial
  ARE Construct 4 - Sense Strand
  misc_feature (1)..(1): n = g + Fluorophore
ngtacagcatgttct

SEQ ID NO: 18 - DNA, 15 bp, Artificial
  ARE Construct 4 - Antisense Strand
  misc_feature (1)..(1): n = a + Quencher
ngaacatgctgtacc

SEQ ID NO: 19 - DNA, 49 bp, Artificial
  ARE Construct 5 - Sense Strand
  misc_feature (1)..(1): n = a + Fluorophore
  misc_feature (24)..(26): n is a, c, g, or t
  misc_feature (49)..(49): n = t + Quencher
nttttatttaatataatggtacannntgttctattatattaaataaaan

SEQ ID NO: 20 - DNA, 15 bp, Artificial
  ARE Construct 5 - Antisense Strand
  misc_feature (7)..(9): n is a, c, g, or t
agaacannntgtacc

SEQ ID NO: 21 - DNA, 45 bp, Artificial
  ARE Construct 6 - Sense Strand
  misc_feature (1)..(1): n = t + Fluorophore
  misc_feature (22)..(24): n is a, c, g, or t
  misc_feature (45)..(45): n = t + Quencher
nttatttaatataatggtacannntgttctattatattaaataan

SEQ ID NO: 22 - DNA, 15 bp, Artificial
  ARE Construct 6 - Antisense Strand
  misc_feature (7)..(9): n is a, c, g, or t
agaacannntgtacc

SEQ ID NO: 23 - DNA, 39 bp, Artificial
  ARE Construct 7 - Sense Strand
  misc_feature (1)..(1): n = a + Fluorophore
  misc_feature (19)..(21): n is a, c, g, or t
  misc_feature (39)..(39): n = t + Quencher
ntttaatataatggtacannntgttctattatattaaan

SEQ ID NO: 24 - DNA, 15 bp, Artificial
  ARE Construct 7 - Antisense Strand
  misc_feature (7)..(9): n is a, c, g, or t
agaacannntgtacc

SEQ ID NO: 25 - DNA, 33 bp, Artificial
  ARE Construct 8 - Sense Strand
  misc_feature (1)..(1): n = t + Fluorophore
  misc_feature (16)..(18): n is a, c, g, or t
  misc_feature (33)..(33): n = a + Quencher
naatataatggtacannntgttctattatattn

SEQ ID NO: 26 - DNA, 15 bp, Artificial
  ARE Construct 8 - Antisense Strand
  misc_feature (7)..(9): n is a, c, g, or t
agaacannntgtacc

SEQ ID NO: 27 - DNA, 27 bp, Artificial
  ARE Construct 9 - Sense Strand
  misc_feature (1)..(1): n = t + Fluorophore
  misc_feature (12)..(15): n is a, c, g, or t
  misc_feature (27)..(27): n = a + Quencher
nataatggtacnnnntgttctattatn

SEQ ID NO: 28 - DNA, 15 bp, Artificial
  ARE Construct 9 - Antisense Strand
  misc_feature (7)..(9): n is a, c, g, or t
agaacannntgtacc

SEQ ID NO: 29 - DNA, 15 bp, Artificial
  ARE Construct 10 - Sense Strand
  misc_feature (6)..(6): n = a + Fluorophore
  misc_feature (7)..(9): n is a, c, g, or t
ggtacnnnntgttct

SEQ ID NO: 30 - DNA, 15 bp, Artificial
  ARE Construct 10 - Antisense Strand
  misc_feature (7)..(9): n is a, c, g, or t
  misc_feature (10)..(10): n = t + Quencher
agaacannnngtacc

SEQ ID NO: 31 - DNA, 15 bp, Artificial
  ARE Construct 11 - Sense Strand
  misc_feature (7)..(9): n is a, c, g, or t
  misc_feature (10)..(10): n = t + Quencher
ggtacannnngttct

SEQ ID NO: 32 - DNA, 15 bp, Artificial
  ARE Construct 11 - Antisense Strand
  misc_feature (6)..(6): n = a + Quencher
  misc_feature (7)..(9): n is a, c, g, or t
agaacnnnntgtacc

SEQ ID NO: 33 - DNA, 15 bp, Artificial
  ARE Construct 12 - Sense Strand
  misc_feature (7)..(9): n is a, c, g, or t
  misc_feature (10)..(10): n = t + Fluorophore
ggtacannnngttct

SEQ ID NO: 34 - DNA, 15 bp, Artificial
  ARE Construct 12 - Antisense Strand
  misc_feature (7)..(9): n is a, c, g, or t
  misc_feature (10)..(10): n = t + Quencher
agaacannnngtacc

SEQ ID NO: 35 - DNA, 30 bp, Artificial
  ARE Construct 13 - Sense Strand
  misc_feature (6)..(6): n = a + Fluorophore
  misc_feature (7)..(9): n is a, c, g, or t
ggtacnnnntgttctggtacagcatgttct

SEQ ID NO: 36 - DNA, 30 bp, Artificial
  ARE Construct 13 - Antisense Strand
  misc_feature (22)..(24): n is a, c, g, or t
  misc_feature (25)..(25): n = t + Quencher
agaacatgctgtaccagaacannnngtacc

SEQ ID NO: 37 - DNA, 30 bp, Artificial
  ARE Construct 14 - Sense Strand
  misc_feature (7)..(9): n is a, c, g, or t
  misc_feature (10)..(10): n = t + Fluorophore
ggtacannnngttctggtacagcatgttct

SEQ ID NO: 38 - DNA, 30 bp, Artificial; identical to SEQ ID NO: 36
  ARE Construct 14 - Antisense Strand
  misc_feature (22)..(24): n is a, c, g, or t
  misc_feature (25)..(25): n = t + Quencher

SEQ ID NO: 39 - DNA, 30 bp, Artificial
  ARE Construct 15 - Sense Strand
  misc_feature (7)..(9): n is a, c, g, or t
  misc_feature (10)..(10): n = t + Fluorophore
ggtacannnngttctggtacaagctgttct

SEQ ID NO: 40 - DNA, 30 bp, Artificial
  ARE Construct 15 - Antisense Strand
  misc_feature (21)..(21): n = a + Quencher
  misc_feature (22)..(24): n is a, c, g, or t
agaacagcttgtaccagaacnnnntgtacc

SEQ ID NO: 41 - DNA, 15 bp, Artificial
  ARE Construct 16 - Sense Strand
  misc_feature (1)..(1): n = a + Fluorophore
  misc_feature (7)..(9): n is a, c, g, or t
ngaacannntgttct

SEQ ID NO: 42 - DNA, 15 bp, Artificial
  ARE Construct 16 - Antisense Strand
  misc_feature (1)..(1): n = a + Fluorophore
  misc_feature (7)..(9): n is a, c, g, or t
ngaacannntgttct

SEQ ID NO: 43 - DNA, 15 bp, Artificial
  ARE Construct 17 - Sense Strand
  misc_feature (1)..(1): n = a + Fluorophore
ngaacagcatgttct

SEQ ID NO: 44 - DNA, 15 bp, Artificial
  ARE Construct 17 - Antisense Strand
  misc_feature (1)..(1): n = a + Fluorophore
ngaacatgctgttct

SEQ ID NO: 45 - DNA, 15 bp, Artificial
  ARE Construct 18 - Sense Strand
  misc_feature (1)..(1): n = a + Fluorophore
  misc_feature (7)..(9): n is a, c, g, or t
ngaacannntgttct

SEQ ID NO: 46 - DNA, 15 bp, Artificial
  ARE Construct 18 - Antisense Strand
  misc_feature (1)..(1): n = a + Quencher
  misc_feature (7)..(9): n is a, c, g, or t
ngaacannntgttct

SEQ ID NO: 47 - DNA, 15 bp, Artificial
  ARE Construct 19 - Sense Strand
  misc_feature (1)..(1): n = a + Fluorophore
ngaacagcatgttct

SEQ ID NO: 48 - DNA, 15 bp, Artificial
  ARE Construct 19 - Antisense Strand
  misc_feature (1)..(1): n = a + Quencher
ngaacatgctgttct

SEQ ID NO: 49 - DNA, 49 bp, Artificial
  ARE Construct 20 - Sense Strand
  misc_feature (1)..(1): n = a + Fluorophore
  misc_feature (24)..(26): n is a, c, g, or t
  misc_feature (49)..(49): n = T + Quencher
nttttatttaatataatagaacannntgttctattatattaaataaaan

SEQ ID NO: 50 - DNA, 15 bp, Artificial
  ARE Construct 20 - Antisense Strand
  misc_feature (7)..(9): n is a, c, g, or t
agaacannntgttct

SEQ ID NO: 51 - DNA, 45 bp, Artificial
  ARE Construct 21 - Sense Strand
  misc_feature (1)..(1): n = t + Fluorophore
  misc_feature (22)..(24): n is a, c, g, or t
  misc_feature (45)..(45): n = a + Quencher
nttatttaatataatagaacannntgttctattatattaaataan

SEQ ID NO: 52 - DNA, 15 bp, Artificial
  ARE Construct 21 - Antisense Strand
  misc_feature (7)..(9): n is a, c, g, or t
agaacannntgttct

SEQ ID NO: 53 - DNA, 39 bp, Artificial
  ARE Construct 22 - Sense Strand
  misc_feature (1)..(1): n = a + Fluorophore
  misc_feature (19)..(21): n is a, c, g, or t
  misc_feature (39)..(39): n = t + Quencher
ntttaatataatagaacannntgttctattatattaaan

SEQ ID NO: 54 - DNA, 15 bp, Artificial
  ARE Construct 22 - Antisense Strand
  misc_feature (7)..(9): n is a, c, g, or t
agaacannntgttct

SEQ ID NO: 55 - DNA, 33 bp, Artificial
  ARE Construct 23 - Sense Strand
  misc_feature (1)..(1): n = t + Fluorophore
  misc_feature (16)..(18): n is a, c, g, or t
  misc_feature (33)..(33): n = a + Quencher
naatataatagaacannntgttctattatattn

SEQ ID NO: 56 - DNA, 15 bp, Artificial
  ARE Construct 23 - Antisense Strand
  misc_feature (7)..(9): n is a, c, g, or t
agaacannntgttct

SEQ ID NO: 57 - DNA, 27 bp, Artificial
  ARE Construct 24 - Sense Strand
  misc_feature (1)..(1): n = t + Fluorophore
  misc_feature (13)..(15): n is a, c, g, or t
  misc_feature (27)..(27): n = a + Quencher
nataatagaacannntgttctattatn

SEQ ID NO: 58 - DNA, 15 bp, Artificial
  ARE Construct 24 - Antisense Strand
  misc_feature (7)..(9): n is a, c, g, or t
agaacannntgttct

SEQ ID NO: 59 - DNA, 15 bp, Artificial
  ARE Construct 25 - Sense Strand
  misc_feature (6)..(6): n = a + Fluorophore
  misc_feature (7)..(9): n is a, c, g, or t
agaacnnnntgttct

SEQ ID NO: 60 - DNA, 15 bp, Artificial
  ARE Construct 25 - Antisense Strand
  misc_feature (7)..(9): n is a, c, g, or t
  misc_feature (10)..(10): n = t + Quencher
agaacannnngttct

SEQ ID NO: 61 - DNA, 15 bp, Artificial
  ARE Construct 26 - Sense Strand
  misc_feature (7)..(9): n is a, c, g, or t
  misc_feature (10)..(10): n = t + Fluorophore
agaacannnngttct

SEQ ID NO: 62 - DNA, 15 bp, Artificial
  ARE Construct 26 - Antisense Strand
  misc_feature (7)..(9): n is a, c, g, or t
  misc_feature (10)..(10): n = t + Quencher
agaacannnngttct

SEQ ID NO: 63 - DNA, 15 bp, Artificial
  ARE Construct 27 - Sense Strand
  misc_feature (7)..(9): n is a, c, g, or t
  misc_feature (10)..(10): n = t + Fluorophore
agaacannnngttct

SEQ ID NO: 64 - DNA, 15 bp, Artificial
  ARE Construct 27 - Antisense Strand
  misc_feature (6)..(6): n = a + Quencher
  misc_feature (7)..(9): n is a, c, g, or t
agaacnnnntgttct

SEQ ID NO: 65 - DNA, 30 bp, Artificial
  ARE Construct 28 - Sense Strand
  misc_feature (6)..(6): n = a + Fluorophore
  misc_feature (7)..(9): n is a, c, g, or t
agaacnnnntgttctagaacagcatgttct

SEQ ID NO: 66 - DNA, 30 bp, Artificial
  ARE Construct 28 - Antisense Strand
  misc_feature (22)..(24): n is a, c, g, or t
  misc_feature (25)..(25): n = t + Quencher
agaacatgctgttctagaacannnngttct

SEQ ID NO: 67 - DNA, 30 bp, Artificial
  ARE Construct 29 - Sense Strand
  misc_feature (7)..(9): n is a, c, g, or t
  misc_feature (10)..(10): n = t + Fluorophore
agaacannnngttctagaacagcatgttct

SEQ ID NO: 68 - DNA, 30 bp, Artificial; identical to SEQ ID NO: 66
  ARE Construct 29 - Antisense Strand
  misc_feature (22)..(24): n is a, c, g, or t
  misc_feature (25)..(25): n = t + Quencher

SEQ ID NO: 69 - DNA, 30 bp, Artificial; identical to SEQ ID NO: 67
  ARE Construct 30 - Sense Strand
  misc_feature (7)..(9): n is a, c, g, or t
  misc_feature (10)..(10): n = t + Fluorophore

SEQ ID NO: 70 - DNA, 30 bp, Artificial
  ARE Construct 30 - Antisense Strand
  misc_feature (21)..(21): n = a + Quencher
  misc_feature (22)..(24): n is a, c, g, or t
agaacatgctgttctagaacnnnntgttct

SEQ ID NO: 71 - DNA, 15 bp, Artificial
  ERE Construct 31 - Sense Strand
  misc_feature (1)..(1): n = a + Fluorophore
  misc_feature (7)..(9): n is a, c, g, or t
nggtcannntgacct

SEQ ID NO: 72 - DNA, 15 bp, Artificial
  ERE Construct 31 - Antisense Strand
  misc_feature (1)..(1): n = a + Fluorophore
  misc_feature (7)..(9): n is a, c, g, or t
nggtcannntgacct

SEQ ID NO: 73 - DNA, 15 bp, Artificial
  ERE Construct 32 - Sense Strand
  misc_feature (1)..(1): n = a + Fluorophore
nggtcagcatgacct

SEQ ID NO: 74 - DNA, 15 bp, Artificial
  ERE Construct 32 - Antisense Strand
  misc_feature (1)..(1): n = a + Fluorophore
nggtcatgctgacct

SEQ ID NO: 75 - DNA, 15 bp, Artificial
  ERE Construct 33 - Sense Strand
  misc_feature (1)..(1): n = a + Fluorophore
  misc_feature (7)..(9): n is a, c, g, or t
nggtcannntgacct

SEQ ID NO: 76 - DNA, 15 bp, Artificial
  ERE Construct 33 - Antisense Strand
  misc_feature (1)..(1): n = a + Quencher
  misc_feature (7)..(9): n is a, c, g, or t
nggtcannntgacct

SEQ ID NO: 77 - DNA, 15 bp, Artificial
  ERE Construct 34 - Sense Strand
  misc_feature (1)..(1): n = a + Fluorophore
nggtcagcatgacct

SEQ ID NO: 78 - DNA, 15 bp, Artificial
  ERE Construct 34 - Antisense Strand
  misc_feature (1)..(1): n = a + Quencher
nggtcatgctgacct

SEQ ID NO: 79 - DNA, 49 bp, Artificial
  ERE Construct 35 - Sense Strand
  misc_feature (1)..(1): n = a + Fluorophore
  misc_feature (24)..(26): n is a, c, g, or t
  misc_feature (49)..(49): n = t + Quencher
nttttatttaatataataggtcannntgacctattatattaaataaaan

SEQ ID NO: 80 - DNA, 15 bp, Artificial
  ERE Construct 35 - Antisense Strand
  misc_feature (7)..(9): n is a, c, g, or t
aggtcannntgacct

SEQ ID NO: 81 - DNA, 45 bp, Artificial
  ERE Construct 36 - Sense Strand
  misc_feature (1)..(1): n = t + Fluorophore
  misc_feature (22)..(24): n is a, c, g, or t
  misc_feature (45)..(45): n = a + Quencher
nttatttaatataataggtcannntgacctattatattaaataan

SEQ ID NO: 82 - DNA, 15 bp, Artificial
  ERE Construct 36 - Antisense Strand
  misc_feature (7)..(9): n is a, c, g, or t
aggtcannntgacct

SEQ ID NO: 83 - DNA, 39 bp, Artificial
  ERE Construct 37 - Sense Strand
  misc_feature (1)..(1): n = a + Fluorophore
  misc_feature (19)..(21): n is a, c, g, or t
  misc_feature (39)..(39): n = t + Quencher
ntttaatataataggtcannntgacctattatattaaan

SEQ ID NO: 84 - DNA, 15 bp, Artificial
  ERE Construct 37 - Antisense Strand
  misc_feature (7)..(9): n is a, c, g, or t
aggtcannntgacct

SEQ ID NO: 85 - DNA, 33 bp, Artificial
  ERE Construct 38 - Sense Strand
  misc_feature (1)..(1): n = t + Fluorophore
  misc_feature (16)..(18): n is a, c, g, or t
  misc_feature (33)..(33): n = a + Quencher
naatataataggtcannntgacctattatattn

SEQ ID NO: 86 - DNA, 15 bp, Artificial
  ERE Construct 38 - Antisense Strand
  misc_feature (7)..(9): n is a, c, g, or t
aggtcannntgacct

SEQ ID NO: 87 - DNA, 27 bp, Artificial
  ERE Construct 39 - Sense Strand
  misc_feature (1)..(1): n = t + Fluorophore
  misc_feature (13)..(15): n is a, c, g, or t
  misc_feature (27)..(27): n = a + Quencher
nataataggtcannntgacctattatn

SEQ ID NO: 88 - DNA, 15 bp, Artificial
  ERE Construct 39 - Antisense Strand
  misc_feature (7)..(9): n is a, c, g, or t
aggtcannntgacct

SEQ ID NO: 89 - DNA, 15 bp, Artificial
  ERE Construct 40 - Sense Strand
  misc_feature (6)..(6): n = a + Fluorophore
  misc_feature (7)..(9): n is a, c, g, or t
aggtcnnnntgacct

SEQ ID NO: 90 - DNA, 15 bp, Artificial
  ERE Construct 40 - Antisense Strand
  misc_feature (7)..(9): n is a, c, g, or t
  misc_feature (10)..(10): n = t + Quencher
aggtcannnngacct

SEQ ID NO: 91 - DNA, 15 bp, Artificial
  ERE Construct 41 - Sense Strand
  misc_feature (7)..(9): n is a, c, g, or t
  misc_feature (10)..(10): n = t + Fluorophore
aggtcannnngacct

SEQ ID NO: 92 - DNA, 15 bp, Artificial
  ERE Construct 41 - Antisense Strand
  misc_feature (7)..(9): n is a, c, g, or t
  misc_feature (10)..(10): n = t + Quencher
aggtcannnngacct

SEQ ID NO: 93 - DNA, 15 bp, Artificial
  ERE Construct 42 - Sense Strand
  misc_feature (7)..(9): n is a, c, g, or t
  misc_feature (10)..(10): n = t + Fluorophore
aggtcannnngacct

SEQ ID NO: 94 - DNA, 15 bp, Artificial
  ERE Construct 42 - Antisense Strand
  misc_feature (6)..(6): n = a + Quencher
  misc_feature (7)..(9): n is a, c, g, or t
aggtcnnnntgacct

SEQ ID NO: 95 - DNA, 30 bp, Artificial
  ERE Construct 43 - Sense Strand
  misc_feature (6)..(6): n = a + Fluorophore
  misc_feature (7)..(9): n is a, c, g, or t
aggtcnnnntgacctaggtcagcatgacct

SEQ ID NO: 96 - DNA, 30 bp, Artificial
  ERE Construct 43 - Antisense Strand
  misc_feature (22)..(24): n is a, c, g, or t
  misc_feature (25)..(25): n = t + Quencher
aggtcatgctgacctaggtcannnngacct

SEQ ID NO: 97 - DNA, 30 bp, Artificial
  ERE Construct 44 - Sense Strand
  misc_feature (7)..(9): n is a, c, g, or t
  misc_feature (10)..(10): n = t + Fluorophore
aggtcannnngacctaggtcagcatgacct

SEQ ID NO: 98 - DNA, 30 bp, Artificial; identical to SEQ ID NO: 96
  ERE Construct 44 - Antisense Strand
  misc_feature (22)..(24): n is a, c, g, or t
  misc_feature (25)..(25): n = t + Quencher

SEQ ID NO: 99 - DNA, 30 bp, Artificial; identical to SEQ ID NO: 97
  ERE Construct 45 - Sense Strand
  misc_feature (7)..(9): n is a, c, g, or t
  misc_feature (10)..(10): n = t + Fluorophore

SEQ ID NO: 100 - DNA, 30 bp, Artificial
  ERE Construct 45 - Antisense Strand
  misc_feature (21)..(21): n = a + Quencher
  misc_feature (22)..(24): n is a, c, g, or t
aggtcatgctgacctaggtcnnnntgacct

SEQ ID NO: 101 - DNA, 15 bp, Artificial
  PRE Construct 46 - Sense Strand
  misc_feature (1)..(1): n = g + Fluorophore
  misc_feature (7)..(9): n is a, c, g, or t
ngtacannntgttct

SEQ ID NO: 102 - DNA, 15 bp, Artificial
  PRE Construct 46 - Antisense Strand
  misc_feature (1)..(1): n = a + Fluorophore
  misc_feature (7)..(9): n is a, c, g, or t
ngaacannntgtacc

SEQ ID NO: 103 - DNA, 14 bp, Artificial
  PRE Construct 47 - Sense Strand
  misc_feature (1)..(1): n = g + Fluorophore
ngtacacatgttct

SEQ ID NO: 104 - DNA, 14 bp, Artificial
  PRE Construct 47 - Antisense Strand
  misc_feature (1)..(1): n = a + Fluorophore
ngaacatgtgtacc

SEQ ID NO: 105 - DNA, 15 bp, Artificial
  PRE Construct 48 - Sense Strand
  misc_feature (1)..(1): n = g + Fluorophore
  misc_feature (7)..(9): n is a, c, g, or t
ngtacannntgttct

SEQ ID NO: 106 - DNA, 15 bp, Artificial
  PRE Construct 48 - Antisense Strand
  misc_feature (1)..(1): n = a + Quencher
  misc_feature (7)..(9): n is a, c, g, or t
ngaacannntgtacc

SEQ ID NO: 107 - DNA, 14 bp, Artificial
  PRE Construct 49 - Sense Strand
  misc_feature (1)..(1): n = g + Fluorophore
ngtacacatgttct

SEQ ID NO: 108 - DNA, 14 bp, Artificial
  PRE Construct 49 - Antisense Strand
  misc_feature (1)..(1): n = a + Quencher
ngaacatgtgtacc

SEQ ID NO: 109 - DNA, 49 bp, Artificial; identical to SEQ ID NO: 19
  PRE Construct 50 - Sense Strand
  misc_feature (1)..(1): n = a + Fluorophore
  misc_feature (24)..(26): n is a, c, g, or t
  misc_feature (49)..(49): n = t + Quencher

SEQ ID NO: 110 - DNA, 15 bp, Artificial
  PRE Construct 50 - Antisense Strand
  misc_feature (7)..(9): n is a, c, g, or t
agaacannntgtacc

SEQ ID NO: 111 - DNA, 45 bp, Artificial; identical to SEQ ID NO: 21
  PRE Construct 51 - Sense Strand
  misc_feature (1)..(1): n = t + Fluorophore
  misc_feature (22)..(24): n is a, c, g, or t
  misc_feature (45)..(45): n = a + Quencher

SEQ ID NO: 112 - DNA, 15 bp, Artificial
  PRE Construct 51 - Antisense Strand
  misc_feature (7)..(9): n is a, c, g, or t
agaacannntgtacc

SEQ ID NO: 113 - DNA, 39 bp, Artificial; identical to SEQ ID NO: 23
  PRE Construct 52 - Sense Strand
  misc_feature (1)..(1): n = a + Fluorophore
  misc_feature (19)..(21): n is a, c, g, or t
  misc_feature (39)..(39): n = t + Quencher

SEQ ID NO: 114 - DNA, 15 bp, Artificial
  PRE Construct 52 - Antisense Strand
  misc_feature (7)..(9): n is a, c, g, or t
agaacannntgtacc

SEQ ID NO: 115 - DNA, 33 bp, Artificial; identical to SEQ ID NO: 25
  PRE Construct 53 - Sense Strand
  misc_feature (1)..(1): n = t + Fluorophore
  misc_feature (16)..(18): n is a, c, g, or t
  misc_feature (33)..(33): n = a + Quencher

SEQ ID NO: 116 - DNA, 15 bp, Artificial
  PRE Construct 53 - Antisense Strand
  misc_feature (7)..(9): n is a, c, g, or t
agaacannntgtacc

SEQ ID NO: 117 - DNA, 27 bp, Artificial
  PRE Construct 54 - Sense Strand
  misc_feature (1)..(1): n = t + Fluorophore
  misc_feature (13)..(15): n is a, c, g, or t
  misc_feature (27)..(27): n = a + Quencher
nataatggtacannntgttctattatn

SEQ ID NO: 118 - DNA, 15 bp, Artificial
  PRE Construct 54 - Antisense Strand
  misc_feature (6)..(9): n is a, c, g, or t
agaacnnnntgtacc

SEQ ID NO: 119 - DNA, 15 bp, Artificial
  PRE Construct 55 - Sense Strand
  misc_feature (6)..(6): n = a + Fluorophore
  misc_feature (7)..(9): n is a, c, g, or t
ggtacnnnntgttct

SEQ ID NO: 120 - DNA, 15 bp, Artificial
  PRE Construct 55 - Antisense Strand
  misc_feature (7)..(9): n is a, c, g, or t
  misc_feature (10)..(10): n = t + Quencher
agaacannnngtacc

SEQ ID NO: 121 - DNA, 15 bp, Artificial
  PRE Construct 56 - Sense Strand
  misc_feature (7)..(9): n is a, c, g, or t
  misc_feature (10)..(10): n = t + Fluorophore
ggtacannnngttct

SEQ ID NO: 122 - DNA, 15 bp, Artificial
  PRE Construct 56 - Antisense Strand
  misc_feature (7)..(9): n is a, c, g, or t
  misc_feature (10)..(10): n = t + Quencher
agaacannnngtacc

SEQ ID NO: 123 - DNA, 15 bp, Artificial
  PRE Construct 57 - Sense Strand
  misc_feature (7)..(9): n is a, c, g, or t
  misc_feature (10)..(10): n = t + Fluorophore
ggtacannnngttct

SEQ ID NO: 124 - DNA, 15 bp, Artificial
  PRE Construct 57 - Antisense Strand
  misc_feature (6)..(6): n = a + Quencher
  misc_feature (7)..(9): n is a, c, g, or t
agaacnnnntgtacc

SEQ ID NO: 125 - DNA, 30 bp, Artificial; identical to SEQ ID NO: 35
  PRE Construct 58 - Sense Strand
  misc_feature (6)..(6): n = a + Fluorophore
  misc_feature (7)..(9): n is a, c, g, or t

SEQ ID NO: 126 - DNA, 30 bp, Artificial; identical to SEQ ID NO: 36
  PRE Construct 58 - Antisense Strand
  misc_feature (22)..(24): n is a, c, g, or t
  misc_feature (25)..(25): n = t + Quencher

SEQ ID NO: 127 - DNA, 30 bp, Artificial; identical to SEQ ID NO: 37
  PRE Construct 59 - Sense Strand
  misc_feature (7)..(9): n is a, c, g, or t
  misc_feature (10)..(10): n = t + Fluorophore

SEQ ID NO: 128 - DNA, 30 bp, Artificial; identical to SEQ ID NO: 36
  PRE Construct 59 - Antisense Strand
  misc_feature (22)..(24): n is a, c, g, or t
  misc_feature (25)..(25): n = t + Quencher

SEQ ID NO: 129 - DNA, 30 bp, Artificial; identical to SEQ ID NO: 37
  PRE Construct 60 - Sense Strand
  misc_feature (7)..(9): n is a, c, g, or t
  misc_feature (10)..(10): n = t + Fluorophore

SEQ ID NO: 130 - DNA, 30 bp, Artificial
  PRE Construct 60 - Antisense Strand
  misc_feature (21)..(21): n = a + Quencher
  misc_feature (22)..(24): n is a, c, g, or t
agaacatgctgtaccagaacnnnntgtacc

SEQ ID NO: 131 - DNA, 15 bp, Artificial
  MRE/GRE Construct 61 - Sense Strand
  misc_feature (1)..(1): n = a + Fluorophore
  misc_feature (7)..(9): n is a, c, g, or t
ngaacannntgttct

SEQ ID NO: 132 - DNA, 15 bp, Artificial
  MRE/GRE Construct 61 - Antisense Strand
  misc_feature (1)..(1): n = a + Fluorophore
  misc_feature (7)..(9): n is a, c, g, or t
ngaacannntgttct

SEQ ID NO: 133 - DNA, 15 bp, Artificial
  MRE/GRE Construct 62 - Sense Strand
  misc_feature (1)..(1): n = a + Fluorophore
ngaacagcatgttct

SEQ ID NO: 134 - DNA, 15 bp, Artificial
  MRE/GRE Construct 62 - Antisense Strand
  misc_feature (1)..(1): n = a + Fluorophore
ngaacatgctgttct

SEQ ID NO: 135 - DNA, 15 bp, Artificial
  MRE/GRE Construct 63 - Sense Strand
  misc_feature (1)..(1): n = a + Fluorophore
  misc_feature (7)..(9): n is a, c, g, or t
ngaacannntgttct

SEQ ID NO: 136 - DNA, 15 bp, Artificial
  MRE/GRE Construct 63 - Antisense Strand
  misc_feature (1)..(1): n = a + Quencher
  misc_feature (7)..(9): n is a, c, g, or t
ngaacannntgttct

SEQ ID NO: 137 - DNA, 15 bp, Artificial
  MRE/GRE Construct 64 - Sense Strand
  misc_feature (1)..(1): n = a + Fluorophore
ngaacagcatgttct

SEQ ID NO: 138 - DNA, 15 bp, Artificial
  MRE/GRE Construct 64 - Antisense Strand
  misc_feature (1)..(1): n = a + Quencher
ngaacatgctgttct

SEQ ID NO: 139 - DNA, 49 bp, Artificial; identical to SEQ ID NO: 49
  MRE/GRE Construct 65 - Sense Strand
  misc_feature (1)..(1): n = a + Fluorophore
  misc_feature (24)..(26): n is a, c, g, or t
  misc_feature (49)..(49): n = t + Quencher

SEQ ID NO: 140 - DNA, 15 bp, Artificial
  MRE/GRE Construct 65 - Antisense Strand
  misc_feature (7)..(9): n is a, c, g, or t
agaacannntgttct

SEQ ID NO: 141 - DNA, 45 bp, Artificial; identical to SEQ ID NO: 51
  MRE/GRE Construct 66 - Sense Strand
  misc_feature (1)..(1): n = t + Fluorophore
  misc_feature (22)..(24): n is a, c, g, or t
  misc_feature (45)..(45): n = a + Quencher

SEQ ID NO: 142 - DNA, 15 bp, Artificial
  MRE/GRE Construct 66 - Antisense Strand
  misc_feature (7)..(9): n is a, c, g, or t
agaacannntgttct

SEQ ID NO: 143 - DNA, 39 bp, Artificial; identical to SEQ ID NO: 53
  MRE/GRE Construct 67 - Sense Strand
  misc_feature (1)..(1): n = a + Fluorophore
  misc_feature (19)..(21): n is a, c, g, or t
  misc_feature (39)..(39): n = t + Quencher

SEQ ID NO: 144 - DNA, 15 bp, Artificial
  MRE/GRE Construct 67 - Antisense Strand
  misc_feature (7)..(9): n is a, c, g, or t
agaacannntgttct

SEQ ID NO: 145 - DNA, 33 bp, Artificial; identical to SEQ ID NO: 55
  MRE/GRE Construct 68 - Sense Strand
  misc_feature (1)..(1): n = t + Fluorophore
  misc_feature (16)..(18): n is a, c, g, or t
  misc_feature (33)..(33): n = a + Quencher

SEQ ID NO: 146 - DNA, 15 bp, Artificial
  MRE/GRE Construct 68 - Antisense Strand
  misc_feature (7)..(9): n is a, c, g, or t
agaacannntgttct

SEQ ID NO: 147 - DNA, 27 bp, Artificial
  MRE/GRE Construct 69 - Sense Strand
  misc_feature (1)..(1): n = t + Fluorophore
  misc_feature (13)..(15): n is a, c, g, or t
  misc_feature (27)..(27): n = A + Quencher
nataatagaacannntgttctattatn

SEQ ID NO: 148 - DNA, 15 bp, Artificial
  MRE/GRE Construct 69 - Antisense Strand
  misc_feature (7)..(9): n is a, c, g, or t
agaacannntgttct

SEQ ID NO: 149 - DNA, 14 bp, Artificial
  MRE/GRE Construct 70 - Sense Strand
  misc_feature (6)..(6): n = a + Fluorophore
  misc_feature (7)..(9): n is a, c, g, or t
agaacnnnntttct

SEQ ID NO: 150 - DNA, 15 bp, Artificial
  MRE/GRE Construct 70 - Antisense Strand
  misc_feature (7)..(9): n is a, c, g, or t
  misc_feature (10)..(10): n = t + Quencher
agaacannnngttct

SEQ ID NO: 151 - DNA, 15 bp, Artificial
  MRE/GRE Construct 71 - Sense Strand
  misc_feature (7)..(9): n is a, c, g, or t
  misc_feature (10)..(10): n = t + Fluorophore
agaacannnngttct

SEQ ID NO: 152 - DNA, 15 bp, Artificial
  MRE/GRE Construct 71 - Antisense Strand
  misc_feature (7)..(9): n is a, c, g, or t
  misc_feature (10)..(10): n = t + Quencher
agaacannnngttct

SEQ ID NO: 153 - DNA, 15 bp, Artificial
  MRE/GRE Construct 72 - Sense Strand
  misc_feature (7)..(9): n is a, c, g, or t
  misc_feature (10)..(10): n = t + Fluorophore
agaacannnngttct

SEQ ID NO: 154 - DNA, 15 bp, Artificial
  MRE/GRE Construct 72 - Antisense Strand
  misc_feature (6)..(6): n = a + Quencher
  misc_feature (7)..(9): n is a, c, g, or t
agaacnnnntgttct

SEQ ID NO: 155 - DNA, 30 bp, Artificial; identical to SEQ ID NO: 65
  MRE/GRE Construct 73 - Sense Strand
  misc_feature (6)..(6): n = a + Fluorophore
  misc_feature (7)..(9): n is a, c, g, or t

SEQ ID NO: 156 - DNA, 30 bp, Artificial; identical to SEQ ID NO: 66
  MRE/GRE Construct 73 - Antisense Strand
  misc_feature (22)..(24): n is a, c, g, or t
  misc_feature (25)..(25): n = t + Quencher

SEQ ID NO: 157 - DNA, 30 bp, Artificial; identical to SEQ ID NO: 67
  MRE/GRE Construct 74 - Sense Strand
  misc_feature (7)..(9): n is a, c, g, or t
  misc_feature (10)..(10): n = t + Fluorophore

SEQ ID NO: 158 - DNA, 30 bp, Artificial; identical to SEQ ID NO: 66
  MRE/GRE Construct 74 - Antisense Strand
  misc_feature (22)..(24): n is a, c, g, or t
  misc_feature (25)..(25): n = t + Quencher

SEQ ID NO: 159 - DNA, 30 bp, Artificial; identical to SEQ ID NO: 67
  MRE/GRE Construct 75 - Sense Strand
  misc_feature (7)..(9): n is a, c, g, or t
  misc_feature (10)..(10): n = t + Fluorophore

SEQ ID NO: 160 - DNA, 30 bp, Artificial; identical to SEQ ID NO: 70
  MRE/GRE Construct 75 - Antisense Strand
  misc_feature (21)..(21): n = a + Quencher
  misc_feature (22)..(24): n is a, c, g, or t

SEQ ID NO: 161 - DNA, 33 bp, Artificial
  ARE/ERE multiplexed assay reporter construct
  misc_feature (7)..(9): n is a, c, g, or t
  misc_feature (16)..(18): n is a, c, g, or t
  misc_feature (25)..(27): n is a, c, g, or t
agaacannntgttctnnnaggtcannntgacct

SEQ ID NO: 162 - DNA, 33 bp, Artificial
  ARE/ERE multiplexed assay reporter construct
  misc_feature (7)..(9): n is a, c, g, or t
  misc_feature (16)..(18): n is a, c, g, or t
  misc_feature (25)..(27): n is a, c, g, or t
aggtcannntgacctnnnagaacannntgttct

SEQ ID NO: 163 - DNA, 33 bp, Artificial
  ARE/ERE Construct 76 - Sense Strand
  misc_feature (1)..(1): n = a + Fluorophore
  misc_feature (7)..(9): n is a, c, g, or t
  misc_feature (16)..(18): n is a, c, g, or t
  misc_feature (25)..(27): n is a, c, g, or t
ngaacannntgttctnnnaggtcannntgacct

SEQ ID NO: 164 - DNA, 33 bp, Artificial
  ARE/ERE Construct 76 - Antisense Strand
  misc_feature (1)..(1): n = a + Fluorophore
  misc_feature (7)..(9): n is a, c, g, or t
  misc_feature (16)..(18): n is a, c, g, or t
  misc_feature (25)..(27): n is a, c, g, or t
nggtcannntgacctnnnagaacannntgttct

SEQ ID NO: 165 - DNA, 33 bp, Artificial
  ARE/ERE Construct 77 - Sense Strand
  misc_feature (1)..(1): n = a + Fluorophore
  misc_feature (16)..(18): n is a, c, g, or t
ngaacagcatgttctnnnaggtcagcatgacct

SEQ ID NO: 166 - DNA, 33 bp, Artificial
  ARE/ERE Construct 77 - Antisense Strand
  misc_feature (1)..(1): n = a + Fluorophore
  misc_feature (16)..(18): n is a, c, g, or t
nggtcatgctgacctnnnagaacatgctgttct

SEQ ID NO: 167 - DNA, 33 bp, Artificial
  ARE/ERE Construct 78 - Sense Strand
  misc_feature (1)..(1): n = a + Fluorophore
  misc_feature (7)..(9): n is a, c, g, or t
  misc_feature (16)..(18): n is a, c, g, or t
  misc_feature (25)..(27): n is a, c, g, or t
ngaacannntgttctnnntccagtnnnactgga

SEQ ID NO: 168 - DNA, 33 bp, Artificial
  ARE/ERE Construct 78 - Antisense Strand
  misc_feature (1)..(1): n = a + Quencher
  misc_feature (7)..(9): n is a, c, g, or t
  misc_feature (16)..(18): n is a, c, g, or t
  misc_feature (25)..(27): n is a, c, g, or t
nccagtnnnactggannnagaacannntgttct

SEQ ID NO: 169 - DNA, 33 bp, Artificial; identical to SEQ ID NO: 165
  ARE/ERE Construct 79 - Sense Strand
  misc_feature (1)..(1): n = a + Fluorophore
  misc_feature (16)..(18): n is a, c, g, or t

SEQ ID NO: 170 - DNA, 33 bp, Artificial; identical to SEQ ID NO: 166
  ARE/ERE Construct 79 - Antisense Strand
  misc_feature (1)..(1): n = a + Quencher
  misc_feature (16)..(18): n is a, c, g, or t

SEQ ID NO: 171 - DNA, 15 bp, Artificial
  Primary ARE + Cy3 - Sense strand
  misc_feature (1)..(1): n = a + Cy3
ngaacagcatgttct

SEQ ID NO: 172 - DNA, 15 bp, Artificial
  Primary ARE + Cy5 - Antisense strand
  misc_feature (1)..(1): n = a + Cy5
ngaacatgctgttct

SEQ ID NO: 173 - DNA, 17 bp, Artificial
  Primary ERE + Cy3 - Sense strand
  misc_feature (1)..(1): n = c + Cy3
naggtcagcatgacctg

SEQ ID NO: 174 - DNA, 17 bp, Artificial
  Primary ERE + Cy5 - Antisense strand
  misc_feature (1)..(1): n = c + Cy5
naggtcatgctgacctg